European Patent Application EP 4 706 689 A2, published March 11, 2026. Title: COMPOSITIONS FOR DELIVERY OF ANTISENSE COMPOUNDS. Applicant: Entrada Therapeutics, Inc. Application EP, filed January 8, 2026. The sequence listing filed with the application follows.

SEQUENCE LISTING (272 sequences)

SEQ ID NO: 1 - protein, 5 aa, synthetic construct
  REGION 1..5: note = Synthetic Construct
  MOD_RES 2: note = L-2-naphthylalanine
FXRRR

SEQ ID NO: 2 - protein, 6 aa, synthetic construct
  REGION 1..6: note = Synthetic Construct
  MOD_RES 2: note = L-2-naphthylalanine
FXRRRC

SEQ ID NO: 3 - protein, 6 aa, synthetic construct
  REGION 1..6: note = Synthetic Construct
  MOD_RES 2: note = L-2-naphthylalanine
  MOD_RES 6: note = Selenocysteine
FXRRRX

SEQ ID NO: 4 - protein, 5 aa, synthetic construct
  REGION 1..5: note = Synthetic Construct
  MOD_RES 4: note = L-2-naphthylalanine
RRRXF

SEQ ID NO: 5 - protein, 6 aa, synthetic construct
  REGION 1..6: note = Synthetic Construct
  MOD_RES 5: note = L-2-naphthylalanine
RRRRXF

SEQ ID NO: 6 - protein, 6 aa, synthetic construct
  REGION 1..6: note = Synthetic Construct
  MOD_RES 2: note = L-2-naphthylalanine
FXRRRR

SEQ ID NO: 7 - protein, 6 aa, synthetic construct
  REGION 1..6: note = Synthetic Construct
  MOD_RES 2: note = D-2-naphthylalanine
  MOD_RES 3: note = D-amino acid
  MOD_RES 5: note = D-amino acid
FXRRRR

SEQ ID NO: 8 - protein, 6 aa, synthetic construct
  REGION 1..6: note = Synthetic Construct
  MOD_RES 2: note = D-2-naphthylalanine
  MOD_RES 3: note = D-amino acid
  MOD_RES 5: note = D-amino acid
FXRRRR

SEQ ID NO: 9 - protein, 6 aa, synthetic construct
  REGION 1..6: note = Synthetic Construct
  MOD_RES 2: note = L-2-naphthylalanine
FXRRRR

SEQ ID NO: 10 - protein, 6 aa, synthetic construct
  REGION 1..6: note = Synthetic Construct
  MOD_RES 1: note = D-amino acid
  MOD_RES 2: note = L-2-naphthylalanine
  MOD_RES 4: note = D-amino acid
  MOD_RES 6: note = D-amino acid
FXRRRR

SEQ ID NO: 11 - protein, 6 aa, synthetic construct
  REGION 1..6: note = Synthetic Construct
  MOD_RES 5: note = L-2-naphthylalanine
RRFRXR

SEQ ID NO: 12 - protein, 6 aa, synthetic construct
  REGION 1..6: note = Synthetic Construct
  MOD_RES 6: note = L-2-naphthylalanine
FRRRRX

SEQ ID NO: 13 - protein, 6 aa, synthetic construct
  REGION 1..6: note = Synthetic Construct
  MOD_RES 1: note = D-amino acid
  MOD_RES 5: note = L-2-naphthylalanine
RRFRXR

SEQ ID NO: 14 - protein, 6 aa, synthetic construct
  REGION 1..6: note = Synthetic Construct
  MOD_RES 3: note = L-2-naphthylalanine
RRXFRR

SEQ ID NO: 15 - protein, 7 aa, synthetic construct
  REGION 1..7: note = Synthetic Construct
CRRRRFW

SEQ ID NO: 16 - protein, 7 aa, synthetic construct
  REGION 1..7: note = Synthetic Construct
  MOD_RES 2: note = D-amino acid
  MOD_RES 3: note = L-2-naphthylalanine
  MOD_RES 5: note = D-amino acid
  MOD_RES 7: note = D-amino acid
FFXRRRR

SEQ ID NO: 17 - protein, 7 aa, synthetic construct
  REGION 1..7: note = Synthetic Construct
  MOD_RES 3: note = L-2-naphthylalanine
FFXRRRR

SEQ ID NO: 18 - protein, 7 aa, synthetic construct
  REGION 1..7: note = Synthetic Construct
  MOD_RES 6: note = L-2-naphthylalanine
RFRFRXR

SEQ ID NO: 19 - protein, 7 aa, synthetic construct
  REGION 1..7: note = Synthetic Construct
  MOD_RES 1: note = Selenocysteine
XRRRRFW

SEQ ID NO: 20 - protein, 7 aa, synthetic construct
  REGION 1..7: note = Synthetic Construct
CRRRRFW

SEQ ID NO: 21 - protein, 8 aa, synthetic construct
  REGION 1..8: note = Synthetic Construct
  MOD_RES 2: note = L-2-naphthylalanine
FXRRRRQK

SEQ ID NO: 22 - protein, 8 aa, synthetic construct
  REGION 1..8: note = Synthetic Construct
  MOD_RES 2: note = L-2-naphthylalanine
FXRRRRQC

SEQ ID NO: 23 - protein, 8 aa, synthetic construct
  REGION 1..8: note = Synthetic Construct
  MOD_RES 1: note = D-amino acid
  MOD_RES 2: note = L-2-naphthylalanine
  MOD_RES 4: note = D-amino acid
  MOD_RES 6: note = D-amino acid
FXRRRRRQ

SEQ ID NO: 24 - protein, 8 aa, synthetic construct
  REGION 1..8: note = Synthetic Construct
  MOD_RES 2: note = L-2-naphthylalanine
FXRRRRRQ

SEQ ID NO: 25 - protein, 9 aa, synthetic construct
  REGION 1..9: note = Synthetic Construct
  MOD_RES 5: note = L-2-naphthylalanine
  MOD_RES 8: note = L-norleucine
RRRRXFDXC

SEQ ID NO: 26 - protein, 5 aa, synthetic construct
  REGION 1..5: note = Synthetic Construct
  MOD_RES 2: note = L-2-naphthylalanine
FXRRR

SEQ ID NO: 27 - protein, 5 aa, synthetic construct
  REGION 1..5: note = Synthetic Construct
FWRRR

SEQ ID NO: 28 - protein, 5 aa, synthetic construct
  REGION 1..5: note = Synthetic Construct
  MOD_RES 4: note = L-2-naphthylalanine
RRRXF

SEQ ID NO: 29 - protein, 5 aa, synthetic construct
  REGION 1..5: note = Synthetic Construct
RRRWF

SEQ ID NO: 30 - protein, 6 aa, synthetic construct
  REGION 1..6: note = Synthetic Construct
  MOD_RES 2: note = L-2-naphthylalanine
FXRRRR

SEQ ID NO: 31 - protein, 5 aa, synthetic construct
  REGION 1..5: note = Synthetic Construct
FFRRR

SEQ ID NO: 32 - protein, 5 aa, synthetic construct
  REGION 1..5: note = Synthetic Construct
  MOD_RES 3: note = D-amino acid
  MOD_RES 5: note = D-amino acid
FFRRR

SEQ ID NO: 33 - protein, 5 aa, synthetic construct
  REGION 1..5: note = Synthetic Construct
  MOD_RES 4: note = D-amino acid
FFRRR

SEQ ID NO: 34 - protein, 5 aa, synthetic construct
  REGION 1..5: note = Synthetic Construct
FRFRR

SEQ ID NO: 35 - protein, 5 aa, synthetic construct
  REGION 1..5: note = Synthetic Construct
FRRFR

SEQ ID NO: 36 - protein, 5 aa, synthetic construct
  REGION 1..5: note = Synthetic Construct
FRRRF

SEQ ID NO: 37 - protein, 5 aa, synthetic construct
  REGION 1..5: note = Synthetic Construct
  MOD_RES 2: note = L-2-naphthylalanine
GXRRR

SEQ ID NO: 38 - protein, 5 aa, synthetic construct
  REGION 1..5: note = Synthetic Construct
FFFRA

SEQ ID NO: 39 - protein, 5 aa, synthetic construct
  REGION 1..5: note = Synthetic Construct
FFFRR

SEQ ID NO: 40 - protein, 6 aa, synthetic construct
  REGION 1..6: note = Synthetic Construct
FFRRRR

SEQ ID NO: 41 - protein, 6 aa, synthetic construct
  REGION 1..6: note = Synthetic Construct
FRRFRR

SEQ ID NO: 42 - protein, 6 aa, synthetic construct
  REGION 1..6: note = Synthetic Construct
FRRRFR

SEQ ID NO: 43 - protein, 6 aa, synthetic construct
  REGION 1..6: note = Synthetic Construct
RFFRRR

SEQ ID NO: 44 - protein, 6 aa, synthetic construct
  REGION 1..6: note = Synthetic Construct
RFRRFR

SEQ ID NO: 45 - protein, 6 aa, synthetic construct
  REGION 1..6: note = Synthetic Construct
FRFRRR

SEQ ID NO: 46 - protein, 6 aa, synthetic construct
  REGION 1..6: note = Synthetic Construct
FFFRRR

SEQ ID NO: 47 - protein, 6 aa, synthetic construct
  REGION 1..6: note = Synthetic Construct
FFRRRF

SEQ ID NO: 48 - protein, 6 aa, synthetic construct
  REGION 1..6: note = Synthetic Construct
FRFFRR

SEQ ID NO: 49 - protein, 6 aa, synthetic construct
  REGION 1..6: note = Synthetic Construct
RRFFFR

SEQ ID NO: 50 - protein, 6 aa, synthetic construct
  REGION 1..6: note = Synthetic Construct
FFRFRR

SEQ ID NO: 51 - protein, 6 aa, synthetic construct
  REGION 1..6: note = Synthetic Construct
FFRRFR

SEQ ID NO: 52 - protein, 6 aa, synthetic construct
  REGION 1..6: note = Synthetic Construct
FRRFFR

SEQ ID NO: 53 - protein, 6 aa, synthetic construct
  REGION 1..6: note = Synthetic Construct
FRRFRF

SEQ ID NO: 54 - protein, 6 aa, synthetic construct
  REGION 1..6: note = Synthetic Construct
FRFRFR

SEQ ID NO: 55 - protein, 6 aa, synthetic construct
  REGION 1..6: note = Synthetic Construct
RFFRFR

SEQ ID NO: 56 - protein, 6 aa, synthetic construct
  REGION 1..6: note = Synthetic Construct
  MOD_RES 2: note = L-2-naphthylalanine
GXRRRR

SEQ ID NO: 57 - protein, 7 aa, synthetic construct
  REGION 1..7: note = Synthetic Construct
FFFRRRR

SEQ ID NO: 58 - protein, 7 aa, synthetic construct
  REGION 1..7: note = Synthetic Construct
RFFRRRR

SEQ ID NO: 59 - protein, 7 aa, synthetic construct
  REGION 1..7: note = Synthetic Construct
RRFFRRR

SEQ ID NO: 60 - protein, 7 aa, synthetic construct
  REGION 1..7: note = Synthetic Construct
RFFFRRR

SEQ ID NO: 61 - protein, 7 aa, synthetic construct
  REGION 1..7: note = Synthetic Construct
RRFFFRR

SEQ ID NO: 62 - protein, 7 aa, synthetic construct
  REGION 1..7: note = Synthetic Construct
FFRRFRR

SEQ ID NO: 63 - protein, 7 aa, synthetic construct
  REGION 1..7: note = Synthetic Construct
FFRRRRF

SEQ ID NO: 64 - protein, 7 aa, synthetic construct
  REGION 1..7: note = Synthetic Construct
FRRFFRR

SEQ ID NO: 65 - protein, 8 aa, synthetic construct
  REGION 1..8: note = Synthetic Construct
FFFRRRRR

SEQ ID NO: 66 - protein, 9 aa, synthetic construct
  REGION 1..9: note = Synthetic Construct
FFFRRRRRR

SEQ ID NO: 67 - protein, 6 aa, synthetic construct
  REGION 1..6: note = Synthetic Construct
  MOD_RES 2: note = L-2-naphthylalanine
  MOD_RES 4: note = D-amino acid
  MOD_RES 6: note = D-amino acid
FXRRRR

SEQ ID NO: 68 - protein, 6 aa, synthetic construct
  REGION 1..6: note = Synthetic Construct
  MOD_RES 1..2: note = L-4-fluorophenylalanine
XXRRRR

SEQ ID NO: 69 - protein, 6 aa, synthetic construct
  REGION 1..6: note = Synthetic Construct
  MOD_RES 2: note = D-amino acid
  MOD_RES 5: note = D-amino acid
FFFRRR

SEQ ID NO: 70 - protein, 6 aa, synthetic construct
  REGION 1..6: note = Synthetic Construct
  MOD_RES 1: note = D-amino acid
  MOD_RES 3..4: note = D-amino acid
  MOD_RES 6: note = D-amino acid
FFFRRR

SEQ ID NO: 71 - protein, 6 aa, synthetic construct
  REGION 1..6: note = Synthetic Construct
  MOD_RES 1: note = D-amino acid
  MOD_RES 3: note = D-amino acid
  MOD_RES 5: note = D-amino acid
FFFRRR

SEQ ID NO: 72 - protein, 6 aa, synthetic construct
  REGION 1..6: note = Synthetic Construct
  MOD_RES 2: note = D-amino acid
  MOD_RES 4: note = D-amino acid
  MOD_RES 6: note = D-amino acid
FFFRRR

SEQ ID NO: 73 - protein, 6 aa, synthetic construct
  REGION 1..6: note = Synthetic Construct
  MOD_RES 1: note = D-amino acid
  MOD_RES 3: note = D-2-naphthylalanine
  MOD_RES 4: note = D-amino acid
  MOD_RES 6: note = D-amino acid
FFXRRR

SEQ ID NO: 74 - protein, 6 aa, synthetic construct
  REGION 1..6: note = Synthetic Construct
  MOD_RES 1: note = D-amino acid
  MOD_RES 2: note = L-2-naphthylalanine
  MOD_RES 3..4: note = D-amino acid
  MOD_RES 6: note = D-amino acid
FXFRRR

SEQ ID NO: 75 - protein, 6 aa, synthetic construct
  REGION 1..6: note = Synthetic Construct
  MOD_RES 1: note = D-2-naphthylalanine
  MOD_RES 3..4: note = D-amino acid
  MOD_RES 6: note = D-amino acid
XFFRRR

SEQ ID NO: 76 - protein, 5 aa, synthetic construct
  REGION 1..5: note = Synthetic Construct
  MOD_RES 2: note = L-2-naphthylalanine
  MOD_RES 3: note = D-amino acid
  MOD_RES 5: note = D-amino acid
FXRRR

SEQ ID NO: 77 - protein, 5 aa, synthetic construct
  REGION 1..5: note = Synthetic Construct
  MOD_RES 1: note = D-amino acid
  MOD_RES 2: note = L-2-naphthylalanine
  MOD_RES 3: note = D-amino acid
  MOD_RES 5: note = D-amino acid
FXRRR

SEQ ID NO: 78 - protein, 8 aa, synthetic construct
  REGION 1..8: note = Synthetic Construct
  MOD_RES 1: note = ACETYLATION
  MOD_RES 2: note = D-amino acid
  MOD_RES 5: note = D-amino acid
  MOD_RES 7: note = D-amino acid
KFFRRRRD

SEQ ID NO: 79 - protein, 8 aa, synthetic construct
  REGION 1..8: note = Synthetic Construct
  MOD_RES 1: note = ACETYLATION
  MOD_RES 1: note = L-2,3-diaminopropionic acid
  MOD_RES 2: note = D-amino acid
  MOD_RES 5: note = D-amino acid
  MOD_RES 7: note = D-amino acid
XFFRRRRD

SEQ ID NO: 80 - protein, 8 aa, synthetic construct
  REGION 1..8: note = Synthetic Construct
  DISULFID 1..8: note = disulfide bond
CWWRRRRC

SEQ ID NO: 81 - protein, 9 aa, synthetic construct
  REGION 1..9: note = Synthetic Construct
  DISULFID 1..9: note = disulfide bond
CWWWRRRRC

SEQ ID NO: 82 - protein, 8 aa, synthetic construct
  REGION 1..8: note = Synthetic Construct
  DISULFID 1..8: note = disulfide bond
CFWRRRRC

SEQ ID NO: 83 - protein, 8 aa, synthetic construct
  REGION 1..8: note = Synthetic Construct
  DISULFID 1..8: note = disulfide bond
CWWWRRRC

SEQ ID NO: 84 - protein, 7 aa, synthetic construct
  REGION 1..7: note = Synthetic Construct
  MOD_RES 1: note = L-homoproline
  MOD_RES 2: note = L-2-naphthylalanine
  MOD_RES 5..7: note = D-amino acid
XXRERRE

SEQ ID NO: 85 - protein, 7 aa, synthetic construct
  REGION 1..7: note = Synthetic Construct
  MOD_RES 1: note = L-homoproline
  MOD_RES 2: note = L-2-naphthylalanine
  MOD_RES 5..7: note = D-amino acid
XXRRRRE

SEQ ID NO: 86 - protein, 7 aa, synthetic construct
  REGION 1..7: note = Synthetic Construct
  MOD_RES 1: note = L-homoproline
  MOD_RES 2..3: note = L-2-naphthylalanine
  MOD_RES 5..7: note = D-amino acid
XXXRRRE

SEQ ID NO: 87 - protein, 7 aa, synthetic construct
  REGION 1..7: note = Synthetic Construct
  MOD_RES 1: note = L-homoproline
  MOD_RES 2..3: note = L-2-naphthylalanine
  MOD_RES 5..6: note = D-amino acid
XXXRRRE

SEQ ID NO: 88 - protein, 7 aa, synthetic construct
  REGION 1..7: note = Synthetic Construct
  MOD_RES 1: note = L-homoproline
  MOD_RES 2: note = L-2-naphthylalanine
  MOD_RES 5..7: note = D-amino acid
XXFRRRE

SEQ ID NO: 89 - protein, 7 aa, synthetic construct
  REGION 1..7: note = Synthetic Construct
  MOD_RES 1: note = L-homoproline
  MOD_RES 2: note = L-2-naphthylalanine
  MOD_RES 5..6: note = D-amino acid
XXFRRRE

SEQ ID NO: 90 - protein, 7 aa, synthetic construct
  REGION 1..7: note = Synthetic Construct
  MOD_RES 1: note = L-homoproline
  MOD_RES 2: note = L-2-naphthylalanine
  MOD_RES 3: note = D-amino acid
  MOD_RES 5..7: note = D-amino acid
XXFRRRE

SEQ ID NO: 91 - protein, 7 aa, synthetic construct
  REGION 1..7: note = Synthetic Construct
  MOD_RES 1: note = L-homoproline
  MOD_RES 2: note = L-2-naphthylalanine
  MOD_RES 3: note = D-amino acid
  MOD_RES 5..6: note = D-amino acid
XXFRRRE

SEQ ID NO: 92 - protein, 7 aa, synthetic construct
  REGION 1..7: note = Synthetic Construct
  MOD_RES 1: note = L-homoproline
  MOD_RES 2: note = L-2-naphthylalanine
  MOD_RES 3: note = D-2-naphthylalanine
  MOD_RES 5..6: note = D-amino acid
XXXRRRE

SEQ ID NO: 93 - protein, 7 aa, synthetic construct
  REGION 1..7: note = Synthetic Construct
  MOD_RES 1: note = L-homoproline
  MOD_RES 2: note = L-2-naphthylalanine
  MOD_RES 3: note = D-2-naphthylalanine
  MOD_RES 5..7: note = D-amino acid
XXXRRRE

SEQ ID NO: 94 - protein, 8 aa, synthetic construct
  REGION 1..8: note = synthetic construct
  MOD_RES 1: note = Arg is modified with pimelic acid
  REGION 1..4: note = MISC_FEATURE - Cyclization between Arg is modified with pimelic acid and Arg is modified with lysine peptoid residue
  MOD_RES 4: note = Arg is modified with lysine peptoid residue
RQRRGRRR

SEQ ID NO: 95 - protein, 19 aa, synthetic construct
  REGION 1..19: note = synthetic construct
  DISULFID 2..19: note = Cys residues jopined by disulfide bond
KCFQWQRNMRKVRGPPVSC

SEQ ID NO: 96 - protein, 11 aa, synthetic construct
  REGION 1..11: note = synthetic construct
  REGION 1..11: note = MISC_FEATURE - Cyclization between Lys and Glu
  MOD_RES 2: note = D-amino acid
  MOD_RES 4: note = D-amino acid
  MOD_RES 6: note = D-amino acid
  MOD_RES 8: note = D-amino acid
  MOD_RES 10: note = D-amino acid
KRRRGRKKRRE

SEQ ID NO: 97 - protein, 12 aa, synthetic construct
  REGION 1..12: note = synthetic construct
  REGION 1..12: note = MISC_FEATURE - Cyclization between Lys and Glu
  MOD_RES 2: note = D-amino acid
  MOD_RES 4: note = D-amino acid
  MOD_RES 6: note = D-amino acid
  MOD_RES 8: note = D-amino acid
  MOD_RES 10: note = D-amino acid
KRRRRRRRRRRE

SEQ ID NO: 98 - protein, 14 aa, synthetic construct
  REGION 1..14: note = synthetic construct
  MOD_RES 13: note = D-amino acid
RVRTRGKRRIRRPP

SEQ ID NO: 99 - protein, 14 aa, synthetic construct
  REGION 1..14: note = synthetic construct
  MOD_RES 13: note = D-amino acid
RTRTRGKRRIRVPP

SEQ ID NO: 100 - protein, 8 aa, synthetic construct
  REGION 1..8: note = synthetic construct
WRWRWRWR

SEQ ID NO: 101 - protein, 34 aa, synthetic construct
  REGION 1..34: note = synthetic construct
  DISULFID 4..21: note = Cys residues jopined by disulfide bond
  DISULFID 11..23: note = Cys residues jopined by disulfide bond
  DISULFID 17..29: note = Cys residues jopined by disulfide bond
GGVCPKILKKCRRDSDCPGACICRGNGYCGSGSD

SEQ ID NO: 102 - protein, 10 aa, synthetic construct
  REGION 1..10: note = synthetic construct
  REGION 1..10: note = MISC_FEATURE - Macrocyclization by multicomponent reaction with aziridine aldehyde and isocyanide
  MOD_RES 2: note = L-3-cyclohexyl-alanine
  MOD_RES 3: note = D-amino acid
  MOD_RES 4: note = L-cyclohexylalanine
  MOD_RES 5: note = D-amino acid
  MOD_RES 6: note = L-cyclohexylalanine
  MOD_RES 7: note = D-amino acid
  MOD_RES 8: note = L-cyclohexylalanine
  MOD_RES 9: note = D-amino acid
PXRXRXRXRG

SEQ ID NO: 103 - protein, 13 aa, synthetic construct
  REGION 1..13: note = synthetic construct
  MOD_RES 1: note = Ser is modified with trimesic acid
  REGION 1..13: note = MISC_FEATURE - N-terminal amine and side chains of two L-2,3-diaminopropionic acid residues bicyclized with trimesic acid
  MOD_RES 2: note = D-amino acid
  MOD_RES 4: note = L-4-(phosphonodifluoromethyl)phenylalanine
  MOD_RES 6: note = L-2,3-diaminopropionic acid
  MOD_RES 8: note = L-naphthylalanine
  MOD_RES 13: note = L-2,3-diaminopropionic acid
SVPXHXFXRRRRX

SEQ ID NO: 104 - protein, 17 aa, synthetic construct
  REGION 1..17: note = synthetic construct
  MOD_RES 1: note = D-alanine is modified with trimesic acid
  MOD_RES 1: note = D-amino acid
  REGION 1..17: note = MISC_FEATURE - N-terminal amine and side chains of two L-2,3-diaminopropionic acid residues bicyclized with trimesic acid
  MOD_RES 2: note = sarcosine
  MOD_RES 4: note = D-phosphothreonine
  MOD_RES 5: note = L-homoproline
  MOD_RES 6: note = L-naphthylalanine
  MOD_RES 9: note = D-alanine
  MOD_RES 10: note = L-2,3-diaminopropionic acid
  MOD_RES 12: note = L-naphthylalanine
  MOD_RES 17: note = L-2,3-diaminopropionic acid
AXDXXXRAXXFXRRRRX

SEQ ID NO: 105 - protein, 16 aa, synthetic construct
  REGION 1..16: note = synthetic construct
  REGION 1..15: note = MISC_FEATURE - Three Cys side chains bicyclized with tris(bromomethyl)benzene
CRRSRRGCGRRSRRCG

SEQ ID NO: 106 - protein, 5 aa, synthetic construct
  REGION 1..5: note = synthetic construct
  REGION 1..2: note = MISC_FEATURE - linked by dodecanoyl moiety
KRRRR

SEQ ID NO: 107 - protein, 16 aa, synthetic construct
  REGION 1..16: note = synthetic construct
LKKLCKLLKKLCKLAG

SEQ ID NO: 108 - protein, 9 aa, synthetic construct
  REGION 1..9: note = synthetic construct
  REGION 5..9: note = MISC_FEATURE - Cyclization between Lys and Glu
RRRRKRRRE

SEQ ID NO: 109 - protein, 9 aa, synthetic construct
  REGION 1..9: note = synthetic construct
  REGION 4..9: note = MISC_FEATURE - Cyclization between Lys and Glu
RRRKRRRRE

SEQ ID NO: 110 - protein, 9 aa, synthetic construct
  REGION 1..9: note = synthetic construct
  REGION 3..9: note = MISC_FEATURE - Cyclization between Lys and Glu
RRKRRRRRE

SEQ ID NO: 111 - protein, 9 aa, synthetic construct
  REGION 1..9: note = synthetic construct
  REGION 2..9: note = MISC_FEATURE - Cyclization between Lys and Glu
RKRRRRRRE

SEQ ID NO: 112 - protein, 8 aa, synthetic construct
  REGION 1..8: note = synthetic construct
CRCRCRCR

SEQ ID NO: 113 - protein, 12 aa, synthetic construct
  REGION 1..12: note = synthetic construct
  MOD_RES 1: note = L-propargylglycine
  REGION 1..12: note = MISC_FEATURE - Cyclization by the click reaction between L-propargylglycine and L-6-Azido-2-amino-hexanoic
  MOD_RES 12: note = L-6-Azido-2-amino-hexanoic
XLRKRLRKFRNX

SEQ ID NO: 114 - protein, 9 aa, synthetic construct
  REGION 1..9: note = synthetic construct
  MOD_RES 2..4: note = L-2,3-diaminopropionic acid
  MOD_RES 5: note = D-amino acid
  MOD_RES 7..8: note = L-2,3-diaminopropionic acid
TXXXFLXXT

SEQ ID NO: 115 - protein, 9 aa, synthetic construct
  REGION 1..9: note = synthetic construct
  MOD_RES 2: note = L-2-amino-3-guanidinylpropionic acid
  MOD_RES 3: note = L-2,3-diaminopropionic acid
  MOD_RES 4: note = L-2-amino-3-guanidinylpropionic acid
  MOD_RES 5: note = D-amino acid
  MOD_RES 7..8: note = L-2-amino-3-guanidinylpropionic acid
TXXXFLXXT

SEQ ID NO: 116 - protein, 6 aa, synthetic construct
  REGION 1..6: note = Synthetic Construct
  MOD_RES 2: note = L-2-naphthylalanine
FXRRRR

SEQ ID NO: 117 - protein, 7 aa, synthetic construct
  REGION 1..7: note = Synthetic Construct
  MOD_RES 2: note = D-amino acid
  MOD_RES 3: note = L-2-naphthylalanine
  MOD_RES 5: note = D-amino acid
  MOD_RES 7: note = D-amino acid
FFXRRRR

SEQ ID NO: 118 - protein, 6 aa, synthetic construct
  REGION 1..6: note = Synthetic Construct
  MOD_RES 1: note = D-amino acid
  MOD_RES 2: note = L-2-naphthylalanine
  MOD_RES 4: note = D-amino acid
  MOD_RES 6: note = D-amino acid
FXRRRR

SEQ ID NO: 119 - protein, 7 aa, synthetic construct
  REGION 1..7: note = Synthetic Construct
  MOD_RES 1: note = D-amino acid
  MOD_RES 2: note = L-2-naphthylalanine
  MOD_RES 4: note = D-amino acid
  MOD_RES 6: note = D-amino acid
FXRRRRR

SEQ ID NO: 120 - protein, 6 aa, synthetic construct
  REGION 1..6: note = Synthetic Construct
  MOD_RES 2: note = D-2-naphthylalanine
  MOD_RES 3: note = D-amino acid
  MOD_RES 5: note = D-amino acid
FXRRRR

SEQ ID NO: 121 - protein, 6 aa, synthetic construct
  REGION 1..6: note = Synthetic Construct
  MOD_RES 2: note = D-2-naphthylalanine
  MOD_RES 3: note = D-amino acid
  MOD_RES 5: note = D-amino acid
FXRRRR

SEQ ID NO: 122 - protein, 7 aa, synthetic construct
  REGION 1..7: note = Synthetic Construct
  MOD_RES 2: note = L-2-naphthylalanine
FXRRRRR

SEQ ID NO: 123 - protein, 7 aa, synthetic construct
  REGION 1..7: note = Synthetic Construct
  MOD_RES 5: note = L-2-naphthylalanine
RRFRXRQ

SEQ ID NO: 124 - protein, 7 aa, synthetic construct
  REGION 1..7: note = Synthetic Construct
  MOD_RES 3: note = L-2-naphthylalanine
FFXRRRR

SEQ ID NO: 125 - protein, 7 aa, synthetic construct
  REGION 1..7: note = Synthetic Construct
  MOD_RES 6: note = L-2-naphthylalanine
RFRFRXR

SEQ ID NO: 126 - protein, 5 aa, synthetic construct
  REGION 1..5: note = Synthetic Construct
  MOD_RES 2: note = L-2-naphthylalanine
FXRRR

SEQ ID NO: 127 - protein, 6 aa, synthetic construct
  REGION 1..6: note = Synthetic Construct
  MOD_RES 6: note = L-2-naphthylalanine
FRRRRX

SEQ ID NO: 128 - protein, 6 aa, synthetic construct
  REGION 1..6: note = Synthetic Construct
  MOD_RES 1: note = D-amino acid
  MOD_RES 5: note = L-2-naphthylalanine
RRFRXR

SEQ ID NO: 129 - protein, 6 aa, synthetic construct
  REGION 1..6: note = Synthetic Construct
  MOD_RES 3: note = L-2-naphthylalanine
RRXFRR

SEQ ID NO: 130 - protein, 6 aa, synthetic construct
  REGION 1..6: note = Synthetic Construct
  MOD_RES 1: note = D-amino acid
  MOD_RES 2: note = L-2-naphthylalanine
  MOD_RES 3..4: note = D-amino acid
  MOD_RES 6: note = D-amino acid
FXFRRR

SEQ ID NO: 131 - protein, 7 aa, synthetic construct
  REGION 1..7: note = nuclear localization sequence
PKKKRKV

SEQ ID NO: 132 - protein, 19 aa, synthetic construct
  REGION 1..19: note = nuclear localization sequence
NLSKRPAAIKKAGQAKKKK

SEQ ID NO: 133 - protein, 9 aa, synthetic construct
  REGION 1..9: note = nuclear localization sequence
PAAKRVKLD

SEQ ID NO: 134 - protein, 11 aa, synthetic construct
  REGION 1..11: note = nuclear localization sequence
RQRRNELKRSF

SEQ ID NO: 135 - protein, 41 aa, synthetic construct
  REGION 1..41: note = nuclear localization sequence
RMRKFKNKGKDTAELRRRRVEVSVELRKAKKDEQILKRRNV

SEQ ID NO: 136 - protein, 8 aa, synthetic construct
  REGION 1..8: note = nuclear localization sequence
VSRKRPRP

SEQ ID NO: 137 - protein, 8 aa, synthetic construct
  REGION 1..8: note = nuclear localization sequence
PPKKARED

SEQ ID NO: 138 - protein, 8 aa, synthetic construct
  REGION 1..8: note = nuclear localization sequence
PQPKKKPL

SEQ ID NO: 139 - protein, 12 aa, synthetic construct
  REGION 1..12: note = nuclear localization sequence
SALIKKKKKMAP

SEQ ID NO: 140 - protein, 5 aa, synthetic construct
  REGION 1..5: note = nuclear localization sequence
DRLRR

SEQ ID NO: 141 - protein, 7 aa, synthetic construct
  REGION 1..7: note = nuclear localization sequence
PKQKKRK

SEQ ID NO: 142 - protein, 10 aa, synthetic construct
  REGION 1..10: note = nuclear localization sequence
RKLKKKIKKL

SEQ ID NO: 143 - protein, 10 aa, synthetic construct
  REGION 1..10: note = nuclear localization sequence
REKKKFLKRR

SEQ ID NO: 144 - protein, 20 aa, synthetic construct
  REGION 1..20: note = nuclear localization sequence
KRKGDEVDGVDEVAKKKSKK

SEQ ID NO: 145 - protein, 17 aa, synthetic construct
  REGION 1..17: note = nuclear localization sequence
RKCLQAGMNLEARKTKK

SEQ ID NO: 146 - protein, 7 aa, synthetic construct
  REGION 1..7: note = synthetic construct
  REGION 1..7: note = MISC_FEATURE - cyclic peptide
  MOD_RES 2: note = L-2-naphthylalanine
FXRRRRQ

SEQ ID NO: 147 - DNA, 16 bp, synthetic construct
  misc_feature 1..16: note = immunostimulatory nucleic acid
  source 1..16: mol_type = other DNA
taacgttgaggggcat

SEQ ID NO: 148 - DNA, 18 bp, synthetic construct
  misc_feature 1..18: note = antisense compound phosphorodiamidate morpholino oligomer (PMO) with a C6-thiol 5' modification
  misc_feature 1: note = C6-thiol 5' modification
  modified_base 1..18: mod_base = OTHER; note = 6 membered morpholine rings replace deoxyribose rings
  modified_base 1..18: mod_base = OTHER; note = linked by non-ionic phosphorodiamidate intersubunit linkages
  source 1..18: mol_type = other DNA
gctattaccttaacccag

SEQ ID NO: 149 - protein, 11 aa, synthetic construct
  REGION 1..11: note = synthetic construct
  MOD_RES 2: note = D-amino acid
  MOD_RES 3: note = L-2-naphthylalanine
  MOD_RES 5: note = D-amino acid
  MOD_RES 7: note = D-amino acid
  MOD_RES 8: note = gamma-glutamate
  MOD_RES 9..10: note = beta-alanine
  MOD_RES 11: note = modiified with maleimide
FFXRRRRXXXK

SEQ ID NO: 150 - DNA, 23 bp, synthetic construct
  misc_feature 1..23: note = RT-PCR primer
  source 1..23: mol_type = other DNA
cgtaaacggccacaagttcagcg

SEQ ID NO: 151 - DNA, 24 bp, synthetic construct
  misc_feature 1..24: note = RT-PCR primer
  source 1..24: mol_type = other DNA
gtggtgcagatgaacttcagggtc

SEQ ID NO: 152 - DNA, 17 bp, synthetic construct
  misc_feature 1..17: note = antisense compound
  source 1..17: mol_type = other DNA
gctattaccttaaccca

SEQ ID NO: 153 - DNA, 21 bp, synthetic construct
  misc_feature 1..21: note = antisense compound
  modified_base 1..21: mod_base = OTHER; note = 6 membered morpholine rings replace deoxyribose rings
  modified_base 1..21: mod_base = OTHER; note = linked by non-ionic phosphorodiamidate intersubunit linkages
  source 1..21: mol_type = other DNA
gtaactgtatttggtacttcc

SEQ ID NO: 154 - DNA, 25 bp, synthetic construct
  misc_feature 1..25: note = antisense compound
  modified_base 1..25: mod_base = OTHER; note = 6 membered morpholine rings replace deoxyribose rings
  misc_feature 1..25: note = linked by non-ionic phosphorodiamidate intersubunit linkages
  misc_feature 25: note = conjugated to CP12 peptide
  source 1..25: mol_type = other DNA
cttcttcttcttcttcttcttcttc

SEQ ID NO: 155 - DNA, 18 bp, synthetic construct
  misc_feature 1..18: note = antisense compound
  misc_feature 1: note = conjugated to CP12 peptide
  modified_base 1..18: mod_base = OTHER; note = 2'-O-MOE ribonucleotides
  misc_feature 1..18: note = linked by phosphorothioate bonds
  source 1..18: mol_type = other DNA
cttcttcttcttcttctt

SEQ ID NO: 156 - DNA, 19 bp, synthetic construct
  misc_feature 1..19: note = antisense compound
  misc_feature 1..19: note = linked by phosphorothioate bonds
  modified_base 1: mod_base = OTHER; note = locked nucleic acid
  misc_feature 1: note = conjugated to CP12 peptide
  modified_base 3..4: mod_base = OTHER; note = locked nucleic acid
  modified_base 6..7: mod_base = OTHER; note = locked nucleic acid
  modified_base 9..10: mod_base = OTHER; note = locked nucleic acid
  modified_base 12..13: mod_base = OTHER; note = locked nucleic acid
  modified_base 15..16: mod_base = OTHER; note = locked nucleic acid
  modified_base 18..19: mod_base = OTHER; note = locked nucleic acid
  source 1..19: mol_type = other DNA
tcttcttcttcttcttctt

SEQ ID NO: 157 - DNA, 18 bp, synthetic construct
  misc_feature 1..18: note = antisense compound
  modified_base 1..18: mod_base = OTHER; note = 6 membered morpholine rings replace deoxyribose rings
  misc_feature 1..18: note = linked by non-ionic phosphorodiamidate intersubunit linkages
  misc_feature 18: note = conjugated to CP12 peptide
  source 1..18: mol_type = other DNA
gctattaccttaacccag

SEQ ID NO: 158 - DNA, 18 bp, synthetic construct
  misc_feature 1..18: note = antisense compound
  modified_base 1..18: mod_base = OTHER; note = 6 membered morpholine rings replace deoxyribose rings
  misc_feature 1..18: note = linked by non-ionic phosphorodiamidate intersubunit linkages
  misc_feature 18: note = conjugated to CP12 peptide and lipid group
  source 1..18: mol_type = other DNA
gctattaccttaacccag

SEQ ID NO: 159 - DNA, 18 bp, synthetic construct
  misc_feature 1..18: note = antisense compound
  modified_base 1..18: mod_base = OTHER; note = 6 membered morpholine rings replace deoxyribose rings
  misc_feature 1..18: note = linked by non-ionic phosphorodiamidate intersubunit linkages
  misc_feature 18: note = conjugated to CP1212 peptide
  source 1..18: mol_type = other DNA
gctattaccttaacccag

SEQ ID NO: 160 - DNA, 18 bp, synthetic construct
  misc_feature 1..18: note = antisense compound
  modified_base 1..18: mod_base = OTHER; note = 6 membered morpholine rings replace deoxyribose rings
  misc_feature 1..18: note = linked by non-ionic phosphorodiamidate intersubunit linkages
  misc_feature 18: note = conjugated to Pip peptide
  source 1..18: mol_type = other DNA
gctattaccttaacccag

SEQ ID NO: 161 - DNA, 24 bp, synthetic construct
  misc_feature 1..24: note = antisense compound
  modified_base 1..24: mod_base = OTHER; note = 6 membered morpholine rings replace deoxyribose rings
  misc_feature 1..24: note = linked by non-ionic phosphorodiamidate intersubunit linkages
  misc_feature 24: note = conjugated to CP12 peptide
  source 1..24: mol_type = other DNA
gggcattttaatatatctctgaac

SEQ ID NO: 162 - DNA, 24 bp, synthetic construct
  misc_feature 1..24: note = antisense compound
  modified_base 1..24: mod_base = OTHER; note = 6 membered morpholine rings replace deoxyribose rings
  misc_feature 1..24: note = linked by non-ionic phosphorodiamidate intersubunit linkages
  misc_feature 24: note = conjugated to CP12 peptide
  source 1..24: mol_type = other DNA
ggccaaacctcggcttacctgaaa

SEQ ID NO: 163 - DNA, 24 bp, synthetic construct
  misc_feature 1..24: note = antisense compound
  modified_base 1..24: mod_base = OTHER; note = 6 membered morpholine rings replace deoxyribose rings
  misc_feature 1..24: note = linked by non-ionic phosphorodiamidate intersubunit linkages
  misc_feature 24: note = conjugated to CP12 peptide and lipid group
  source 1..24: mol_type = other DNA
ggccaaacctcggcttacctgaaa

SEQ ID NO: 164 - DNA, 21 bp, synthetic construct
  misc_feature 1..21: note = antisense compound
  modified_base 1..21: mod_base = OTHER; note = 6 membered morpholine rings replace deoxyribose rings
  misc_feature 1..21: note = linked by non-ionic phosphorodiamidate intersubunit linkages
  misc_feature 21: note = conjugated to CP12 peptide
  source 1..21: mol_type = other DNA
gtaactgtatttggtacttcc

SEQ ID NO: 165 - DNA, 25 bp, synthetic construct
  misc_feature 1..25: note = antisense compound
  modified_base 1..25: mod_base = OTHER; note = 6 membered morpholine rings replace deoxyribose rings
  misc_feature 1..25: note = linked by non-ionic phosphorodiamidate intersubunit linkages
  source 1..25: mol_type = other DNA
ccaactgtcctcaaaagcaggaata

SEQ ID NO: 166 - DNA, 25 bp, synthetic construct
  misc_feature 1..25: note = antisense compound
  modified_base 1..25: mod_base = OTHER; note = 6 membered morpholine rings replace deoxyribose rings
  misc_feature 1..25: note = linked by non-ionic phosphorodiamidate intersubunit linkages
  source 1..25: mol_type = other DNA
ccgggtctgccgcccgctccgccct

SEQ ID NO: 167 - DNA, 18 bp, synthetic construct
  misc_feature 1..18: note = antisense oligonucleotide
  modified_base 1..18: mod_base = OTHER; note = 2'-O-MOE ribonucleotides
  misc_feature 1..18: note = linked by phosphorothioate bonds
  modified_base 3: mod_base = OTHER; note = 5-methyl cytosine
  modified_base 6: mod_base = OTHER; note = 5-methyl cytosine
  modified_base 9: mod_base = OTHER; note = 5-methyl cytosine
  modified_base 12: mod_base = OTHER; note = 5-methyl cytosine
  modified_base 15: mod_base = OTHER; note = 5-methyl cytosine
  modified_base 18: mod_base = OTHER; note = 5-methyl cytosine
  source 1..18: mol_type = other DNA
ttcttcttcttcttcttc

SEQ ID NO: 168 - DNA, 20 bp, synthetic construct
  misc_feature 1..20: note = antisense oligonucleotide
  misc_feature 1..20: note = linked by phosphorothioate bonds
  modified_base 1..4: mod_base = OTHER; note = 2'-O-MOE ribonucleotides
  modified_base 1: mod_base = OTHER; note = 5-methyl cytosine
  modified_base 4: mod_base = OTHER; note = 5-methyl cytosine
  modified_base 7: mod_base = OTHER; note = 5-methyl cytosine
  modified_base 10: mod_base = OTHER; note = 5-methyl cytosine
  modified_base 13: mod_base = OTHER; note = 5-methyl cytosine
  modified_base 16..20: mod_base = OTHER; note = 2'-O-MOE ribonucleotides
  modified_base 16: mod_base = OTHER; note = 5-methyl cytosine
  modified_base 19: mod_base = OTHER; note = 5-methyl cytosine
  source 1..20: mol_type = other DNA
cttcttcttcttcttcttct

SEQ ID NO: 169 - DNA, 20 bp, synthetic construct
  misc_feature 1..20: note = antisense oligonucleotide
  misc_feature 1..20: note = linked by phosphorothioate bonds
  modified_base 1..5: mod_base = OTHER; note = 2'-O-MOE ribonucleotides
  modified_base 2: mod_base = OTHER; note = 5-methyl cytosine
  modified_base 5: mod_base = OTHER; note = 5-methyl cytosine
  modified_base 16..20: mod_base = OTHER; note = 2'-O-MOE ribonucleotides
  modified_base 17: mod_base = OTHER; note = 5-methyl cytosine
  modified_base 20: mod_base = OTHER; note = 5-methyl cytosine
  source 1..20: mol_type = other DNA
tcttcttcttcttcttcttc

SEQ ID NO: 170 - RNA, 19 nt, synthetic construct
  misc_feature 1..19: note = antisense oligonucleotide
  misc_feature 1..4: note = linked by phosphorothioate bonds
  modified_base 1..19: mod_base = OTHER; note = 2'-fluoro ribonucleotides
  misc_feature 17..19: note = linked by phosphorothioate bonds
  source 1..19: mol_type = other RNA
gaagaagaagaagaagaag

SEQ ID NO: 171 - RNA, 19 nt, synthetic construct
  misc_feature 1..19: note = antisense oligonucleotide
  misc_feature 1..3: note = linked by phosphorothioate bonds
  modified_base 1..19: mod_base = OTHER; note = 2'-fluoro ribonucleotides
  misc_feature 16..19: note = linked by phosphorothioate bonds
  source 1..19: mol_type = other RNA
cttcttcttcttcttcttc

SEQ ID NO: 172 - RNA, 19 nt, synthetic construct
  misc_feature 1..19: note = antisense oligonucleotide
  misc_feature 1..4: note = linked by phosphorothioate bonds
  misc_feature 1: note = conjugated to CPP12
  modified_base 1: mod_base = OTHER; note = amidated
  modified_base 1..19: mod_base = OTHER; note = 2'-fluoro ribonucleotides
  misc_feature 17..19: note = linked by phosphorothioate bonds
  source 1..19: mol_type = other RNA
gaagaagaagaagaagaag

SEQ ID NO: 173 - RNA, 19 nt, synthetic construct
  misc_feature 1..19: note = antisense oligonucleotide
  misc_feature 1..3: note = linked by phosphorothioate bonds
  modified_base 1..19: mod_base = OTHER; note = 2'-fluoro ribonucleotides
  misc_feature 16..19: note = linked by phosphorothioate bonds
  source 1..19: mol_type = other RNA
cttcttcttcttcttcttc

SEQ ID NO: 174 - RNA, 19 nt, synthetic construct
  misc_feature 1..19: note = antisense oligonucleotide
  modified_base 1..19: mod_base = OTHER; note = 2'-fluoro ribonucleotides
  misc_feature 17..19: note = linked by phosphorothioate bonds
  modified_base 19: mod_base = OTHER; note = amidated
  misc_feature 19: note = conjugated to CPP12
  source 1..19: mol_type = other RNA
gaagaagaagaagaagaag

SEQ ID NO: 175 - RNA, 19 nt, synthetic construct
  misc_feature 1..19: note = antisense oligonucleotide
  misc_feature 1..3: note = linked by phosphorothioate bonds
  modified_base 1..19: mod_base = OTHER; note = 2'-fluoro ribonucleotides
  misc_feature 16..19: note = linked by phosphorothioate bonds
  source 1..19: mol_type = other RNA
cttcttcttcttcttcttc

SEQ ID NO: 176 - DNA, 21 bp, synthetic construct
  misc_feature 1..21: note = antisense oligonucleotide
  modified_base 1..19: mod_base = OTHER; note = ribonucleotides
  source 1..21: mol_type = other DNA
gaagaagaagaagaagaagtt

SEQ ID NO: 177 - DNA, 21 bp, synthetic construct
  misc_feature 1..21: note = antisense oligonucleotide
  modified_base 1..19: mod_base = OTHER; note = ribonucleotides
  source 1..21: mol_type = other DNA
cttcttcttcttcttcttctt

SEQ ID NO: 178 - DNA, 21 bp, synthetic construct
  misc_feature 1..21: note = antisense oligonucleotide
  modified_base 1..19: mod_base = OTHER; note = ribonucleotides
  source 1..21: mol_type = other DNA
gctataccagcgtcgtcattt

SEQ ID NO: 179 - DNA, 21 bp, synthetic construct
  misc_feature 1..21: note = antisense oligonucleotide
  modified_base 1..19: mod_base = OTHER; note = ribonucleotides
  source 1..21: mol_type = other DNA
atgacgacgctggtatagctt

SEQ ID NO: 180 - DNA, 21 bp, synthetic construct
  misc_feature 1..21: note = antisense oligonucleotide
  modified_base 1..19: mod_base = OTHER; note = ribonucleotides
  source 1..21: mol_type = other DNA
gagtgtctatttgatgaattt

SEQ ID NO: 181 - DNA, 21 bp, synthetic construct
  misc_feature 1..21: note = antisense oligonucleotide
  modified_base 1..19: mod_base = OTHER; note = ribonucleotides
  source 1..21: mol_type = other DNA
attcatcaaatagacactctt

SEQ ID NO: 182 - DNA, 17 bp, synthetic construct
  misc_feature 1..17: note = antisense oligonucleotide
  modified_base 1..17: mod_base = OTHER; note = 2'-O-MOE ribonucleotides
  modified_base 1..2: mod_base = OTHER; note = 5-methyl cytosine
  misc_feature 1..17: note = linked by phosphorothioate bonds
  modified_base 4: mod_base = OTHER; note = 5-methyl cytosine
  modified_base 10: mod_base = OTHER; note = 5-methyl cytosine
  source 1..17: mol_type = other DNA
cctcaaaagcaggaata

SEQ ID NO: 183 - DNA, 15 bp, synthetic construct
  misc_feature 1..15: note = antisense oligonucleotide
  misc_feature 1..15: note = linked by phosphorothioate bonds
  modified_base 1..15: mod_base = OTHER; note = 2'-O-MOE ribonucleotides
  modified_base 1..2: mod_base = OTHER; note = 5-methyl cytosine
  modified_base 7: mod_base = OTHER; note = 5-methyl cytosine
  modified_base 10..11: mod_base = OTHER; note = 5-methyl cytosine
  modified_base 13..15: mod_base = OTHER; note = 5-methyl cytosine
  source 1..15: mol_type = other DNA
ccgggtctgccgccc

SEQ ID NO: 184 - DNA, 17 bp, synthetic construct
  misc_feature 1..17: note = antisense oligonucleotide
  modified_base 1..17: mod_base = OTHER; note = 6 membered morpholine rings replace deoxyribose rings
  misc_feature 1..17: note = linked by non-ionic phosphorodiamidate intersubunit linkages
  source 1..17: mol_type = other DNA
cctcaaaagcaggaata

SEQ ID NO: 185 - DNA, 15 bp, synthetic construct
  misc_feature 1..15: note = antisense oligonucleotide
  modified_base 1..15: mod_base = OTHER; note = 6 membered morpholine rings replace deoxyribose rings
  misc_feature 1..15: note = linked by non-ionic phosphorodiamidate intersubunit linkages
  source 1..15: mol_type = other DNA
ccgggtctgccgccc

SEQ ID NO: 186 - DNA, 25 bp, synthetic construct
  misc_feature 1..25: note = antisense oligonucleotide
  modified_base 1..25: mod_base = OTHER; note = 6 membered morpholine rings replace deoxyribose rings
  misc_feature 1..25: note = linked by non-ionic phosphorodiamidate intersubunit linkages
  source 1..25: mol_type = other DNA
ccaactgtcctcaaaagcaggaata

SEQ ID NO: 187 - DNA, 25 bp, synthetic construct
  misc_feature 1..25: note = antisense oligonucleotide
  modified_base 1..25: mod_base = OTHER; note = 6 membered morpholine rings replace deoxyribose rings
  misc_feature 1..25: note = linked by non-ionic phosphorodiamidate intersubunit linkages
  source 1..25: mol_type = other DNA
ccgggtctgccgcccgctccgccct

SEQ ID NO: 188 - DNA, 25 bp, synthetic construct
  misc_feature 1..25: note = antisense oligonucleotide
  modified_base 1..25: mod_base = OTHER; note = 6 membered morpholine rings replace deoxyribose rings
  misc_feature 1..25: note = linked by non-ionic phosphorodiamidate intersubunit linkages
  source 1..25: mol_type = other DNA
cttcttcttcttcttcttcttcttc

SEQ ID NO: 189 - DNA, 18 bp, synthetic construct
  misc_feature 1..18: note = antisense oligonucleotide
  modified_base 1..18: mod_base = OTHER; note = 2'-O-MOE ribonucleotides
  misc_feature 1..18: note = linked by phosphorothioate bonds
  source 1..18: mol_type = other DNA
cttcttcttcttcttctt

SEQ ID NO: 190 - DNA, 19 bp, synthetic construct
  misc_feature 1..19: note = antisense oligonucleotide
  misc_feature 1..19: note = linked by phosphorothioate bonds
  modified_base 1: mod_base = OTHER; note = locked nucleic acid
  modified_base 3..4: mod_base = OTHER; note = locked nucleic acid
  modified_base 6..7: mod_base = OTHER; note = locked nucleic acid
  modified_base 9..10: mod_base = OTHER; note = locked nucleic acid
  modified_base 12..13: mod_base = OTHER; note = locked nucleic acid
  modified_base 15..16: mod_base = OTHER; note = locked nucleic acid
  modified_base 18..19: mod_base = OTHER; note = locked nucleic acid
  source 1..19: mol_type = other DNA
tcttcttcttcttcttctt

SEQ ID NO: 191 - DNA, 20 bp, synthetic construct
  misc_feature 1..20: note = antisense oligonucleotide
  misc_feature 1..20: note = linked by phosphorothioate bonds
  modified_base 1..5: mod_base = OTHER; note = 2'-O-MOE ribonucleotides
  modified_base 16..20: mod_base = OTHER; note = 2'-O-MOE ribonucleotides
  source 1..20: mol_type = other DNA
cttcttcttcttcttcttct

SEQ ID NO: 192 - DNA, 20 bp, synthetic construct
  misc_feature 1..20: note = antisense oligonucleotide
  misc_feature 1..20: note = linked by phosphorothioate bonds
  modified_base 1..5: mod_base = OTHER; note = 2'-O-MOE ribonucleotides
  modified_base 16..20: mod_base = OTHER; note = 2'-O-MOE ribonucleotides
  source 1..20: mol_type = other DNA
tcttcttcttcttcttcttc

SEQ ID NO: 193 - DNA, 18 bp, synthetic construct
  misc_feature 1..18: note = antisense oligonucleotide
  misc_feature 1..18: note = linked by phosphorothioate bonds
  modified_base 1..18: mod_base = OTHER; note = 2'-O-MOE ribonucleotides
  source 1..18: mol_type = other DNA
cttcttcttcttcttctt

SEQ ID NO: 194 - DNA, 20 bp, synthetic construct
  misc_feature 1..20: note = antisense oligonucleotide
  misc_feature 1..20: note = linked by phosphorothioate bonds
  modified_base 1: mod_base = OTHER; note = modifed with an alkyne moiety
  modified_base 1..5: mod_base = OTHER; note = 2'-O-MOE ribonucleotides
  modified_base 16..20: mod_base = OTHER; note = 2'-O-MOE ribonucleotides
  modified_base 20: mod_base = OTHER; note = modified with a primary amine moiety
  source 1..20: mol_type = other DNA
acagacaataaataccgagg

SEQ ID NO: 195 - DNA, 20 bp, synthetic construct
  misc_feature 1..20: note = antisense oligonucleotide
  misc_feature 1..20: note = linked by phosphorothioate bonds
  modified_base 1: mod_base = OTHER; note = modified with a cycloctyne moiety
  modified_base 1..5: mod_base = OTHER; note = 2'-O-MOE ribonucleotides
  modified_base 16..20: mod_base = OTHER; note = 2'-O-MOE ribonucleotides
  modified_base 20: mod_base = OTHER; note = modified with a primary amine moiety
  source 1..20: mol_type = other DNA
acagacaataaataccgagg

SEQ ID NO: 196 - DNA, 20 bp, synthetic construct
  misc_feature 1..20: note = antisense oligonucleotide
  misc_feature 1..20: note = linked by phosphorothioate bonds
  modified_base 1..5: mod_base = OTHER; note = 2'-O-MOE ribonucleotides
  modified_base 16..20: mod_base = OTHER; note = 2'-O-MOE ribonucleotides
  modified_base 20: mod_base = OTHER; note = modified with a primary amine moiety
  source 1..20: mol_type = other DNA
acagacaataaataccgagg

SEQ ID NO: 197 - DNA, 16 bp, synthetic construct
  misc_feature 1..16: note = antisense oligonucleotide
  misc_feature 1..16: note = linked by phosphorothioate bonds
  modified_base 1: mod_base = OTHER; note = modified with a cyclooctyne moiety
  modified_base 1..3: mod_base = OTHER; note = S-constrained ethyl motif backboned residues
  modified_base 14..16: mod_base = OTHER; note = S-constrained ethyl motif backboned residues
  modified_base 16: mod_base = OTHER; note = modified with a primary amine moiety
  source 1..16: mol_type = other DNA
acaataaataccgagg

SEQ ID NO: 198 - DNA, 16 bp, synthetic construct
  misc_feature 1..16: note = antisense oligonucleotide
  misc_feature 1..16: note = linked by phosphorothioate bonds
  modified_base 1: mod_base = OTHER; note = modified with a cyclooctyne moiety
  modified_base 1..3: mod_base = OTHER; note = S-constrained ethyl motif backboned residues
  modified_base 14..16: mod_base = OTHER; note = S-constrained ethyl motif backboned residues
  misc_feature 16: note = conjugated to CP12 peptide
  source 1..16: mol_type = other DNA
acaataaataccgagg

SEQ ID NO: 199 - DNA, 20 bp, synthetic construct
  misc_feature 1..20: note = antisense oligonucleotide
  misc_feature 1..20: note = linked by phosphorothioate bonds
  modified_base 1..5: mod_base = OTHER; note = 2'-O-MOE ribonucleotides
  modified_base 16..20: mod_base = OTHER; note = 2'-O-MOE ribonucleotides
  modified_base 20: mod_base = OTHER; note = modified with a primary amine moiety
  source 1..20: mol_type = other DNA
cggagcggttgtgaactggc

SEQ ID NO: 200 - DNA, 20 bp, synthetic construct
  misc_feature 1..20: note = antisense oligonucleotide
  misc_feature 1..20: note = linked by phosphorothioate bonds
  modified_base 1: mod_base = OTHER; note = modified with an alkyne moiety
  modified_base 1..5: mod_base = OTHER; note = 2'-O-MOE ribonucleotides
  modified_base 16..20: mod_base = OTHER; note = 2'-O-MOE ribonucleotides
  modified_base 20: mod_base = OTHER; note = modified with a primary amine moiety
  source 1..20: mol_type = other DNA
cggagcggtgtgaactggca

SEQ ID NO: 201 - DNA, 20 bp, synthetic construct
  misc_feature 1..20: note = antisense oligonucleotide
  misc_feature 1..20: note = linked by phosphorothioate bonds
  modified_base 1..5: mod_base = OTHER; note = 2'-O-MOE ribonucleotides
  modified_base 16..20: mod_base = OTHER; note = 2'-O-MOE ribonucleotides
  source 1..20: mol_type = other DNA
acagacaataaataccgagg

SEQ ID NO: 202 - DNA, 20 bp, synthetic construct
  misc_feature 1..20: note = antisense oligonucleotide
  misc_feature 1..20: note = linked by phosphorothioate bonds
  modified_base 1: mod_base = OTHER; note = modified with a alkyne moiety
  modified_base 1..5: mod_base = OTHER; note = 2'-O-MOE ribonucleotides
  modified_base 16..20: mod_base = OTHER; note = 2'-O-MOE ribonucleotides
  misc_feature 20: note = conjugated to a CPP12 peptide through a PEG12 moiety
  source 1..20: mol_type = other DNA
acagacaataaataccgagg

SEQ ID NO: 203 - DNA, 20 bp, synthetic construct
  misc_feature 1..20: note = antisense oligonucleotide
  misc_feature 1..20: note = linked by phosphorothioate bonds
  misc_feature 1: note = conjugated to a CPP12 peptide through a Peg12-Lys-click moiety
  modified_base 1..5: mod_base = OTHER; note = 2'-O-MOE ribonucleotides
  modified_base 16..20: mod_base = OTHER; note = 2'-O-MOE ribonucleotides
  source 1..20: mol_type = other DNA
acagacaataaataccgagg

SEQ ID NO: 204 - DNA, 20 bp, synthetic construct
  misc_feature 1..20: note = antisense oligonucleotide
  misc_feature 1..20: note = linked by phosphorothioate bonds
  misc_feature 1: note = conjugated the a CPP12 peptide through a PEG12-click moiety
  modified_base 1..5: mod_base = OTHER; note = 2'-O-MOE ribonucleotides
  modified_base 16..20: mod_base = OTHER; note = 2'-O-MOE ribonucleotides
  source 1..20: mol_type = other DNA
acagacaataaataccgagg

SEQ ID NO: 205 - DNA, 20 bp, synthetic construct
  misc_feature 1..20: note = antisense oligonucleotide
  misc_feature 1..20: note = linked by phosphorothioate bonds
  misc_feature 1: note = conjugated to a aCPP12-K(CPP12) peptide through a PEG12-K-click moiety
  modified_base 1..5: mod_base = OTHER; note = 2'-O-MOE ribonucleotides
  modified_base 16..20: mod_base = OTHER; note = 2'-O-MOE ribonucleotides
  modified_base 20: mod_base = OTHER; note = modified with a primary amine moiety
  source 1..20: mol_type = other DNA
acagacaataaataccgagg

SEQ ID NO: 206 - DNA, 20 bp, synthetic construct
  misc_feature 1..20: note = antisense oligonucleotide
  misc_feature 1..20: note = linked by phosphorothioate bonds
  misc_feature 1: note = conjugated to Ac-NLS-Lys(CPP12) peptide through a PEG12-K-click moiety
  modified_base 1..5: mod_base = OTHER; note = 2'-O-MOE ribonucleotides
  modified_base 16..20: mod_base = OTHER; note = 2'-O-MOE ribonucleotides
  source 1..20: mol_type = other DNA
acagacaataaataccgagg

SEQ ID NO: 207 - DNA, 20 bp, synthetic construct
  misc_feature 1..20: note = antisense oligonucleotide
  misc_feature 1..20: note = linked by phosphorothioate bonds
  modified_base 1..5: mod_base = OTHER; note = 2'-O-MOE ribonucleotides
  modified_base 16..20: mod_base = OTHER; note = 2'-O-MOE ribonucleotides
  modified_base 20: mod_base = OTHER; note = modified with a primary amine + SMCC moiety
  source 1..20: mol_type = other DNA
acagacaataaataccgagg

SEQ ID NO: 208 - DNA, 21 bp, synthetic construct
  misc_feature 1..21: note = antisense oligonucleotide
  modified_base 1..21: mod_base = OTHER; note = 6 membered morpholine rings replace deoxyribose rings
  misc_feature 1..21: note = linked by non-ionic phosphorodiamidate intersubunit linkages
  modified_base 21: mod_base = OTHER; note = amidated
  source 1..21: mol_type = other DNA
cagcagcagcagcagcagcag

SEQ ID NO: 209 - DNA, 21 bp, synthetic construct
  misc_feature 1..21: note = antisense oligonucleotide
  modified_base 1..21: mod_base = OTHER; note = 6 membered morpholine rings replace deoxyribose rings
  misc_feature 1..21: note = linked by non-ionic phosphorodiamidate intersubunit linkages
  misc_feature 21: note = conjugated to CP12 peptides
  source 1..21: mol_type = other DNA
cagcagcagcagcagcagcag

SEQ ID NO: 210 - DNA, 20 bp, synthetic construct
  misc_feature 1..20: note = antisense oligonucleotide
  misc_feature 1..20: note = linked by phosphorothioate bonds
  modified_base 1: mod_base = OTHER; note = modified with an alkyne moiety
  modified_base 1..5: mod_base = OTHER; note = 2'-O-MOE ribonucleotides
  modified_base 16..20: mod_base = OTHER; note = 2'-O-MOE ribonucleotides
  modified_base 20: mod_base = OTHER; note = modified with a primary amine moiety
  source 1..20: mol_type = other DNA
acagacaataaataccgagg

SEQ ID NO: 211 - DNA, 20 bp, synthetic construct
  misc_feature 1..20: note = antisense oligonucleotide
  misc_feature 1..20: note = linked by phosphorothioate bonds
  modified_base 1..5: mod_base = OTHER; note = 2'-O-MOE ribonucleotides
  modified_base 16..20: mod_base = OTHER; note = 2'-O-MOE ribonucleotides
  modified_base 20: mod_base = OTHER; note = modified with a primary amine moiety
  source 1..20: mol_type = other DNA
cggagcggttgtgaactggc

SEQ ID NO: 212 - DNA, 18 bp, synthetic construct
  misc_feature 1..18: note = antisense oligonucleotide
  source 1..18: mol_type = other DNA
ccataataaagggctcag

SEQ ID NO: 213 - DNA, 20 bp, synthetic construct
  misc_feature 1..20: note = antisense oligonucleotide
  source 1..20: mol_type = other DNA
cagctggagtttatcttttg

SEQ ID NO: 214 - DNA, 24 bp, synthetic construct
  misc_feature 1..24: note = antisense oligonucleotide
  source 1..24: mol_type = other DNA
ggccaaacctcggcttacctgaaa

SEQ ID NO: 215 - RNA, 20 nt, synthetic construct
  misc_feature 1..20: note = exemplary RNA sequence
  source 1..20: mol_type = other RNA
aagaagaagaagaagaagaa

SEQ ID NO: 216 - RNA, 24 nt, synthetic construct
  misc_feature 1..24: note = exemplary RNA sequence
  source 1..24: mol_type = other RNA
aagaagaagaagaagaagaagaag

SEQ ID NO: 217 - DNA, 17 bp, synthetic construct
  misc_feature 1..17: note = antisense oligonucleotide
  misc_feature 1: note = May be conjugated to a chemical moiety
  misc_feature 17: note = May be conjugated to a chemical moiety
  source 1..17: mol_type = other DNA
gctattaccttaaccca

SEQ ID NO: 218 - DNA, 24 bp, synthetic construct
  misc_feature 1..24: note = antisense oligonucleotide
  misc_feature 1: note = May be conjugated to a chemical moiety
  misc_feature 24: note = May be conjugated to a chemical moiety
  source 1..24: mol_type = other DNA
ggccaaacctcggcttacctgaaa

SEQ ID NO: 219 - DNA, 20 bp, synthetic construct
  misc_feature 1..20: note = antisense oligonucleotide
  misc_feature 1: note = May be conjugated to a chemical moiety
  misc_feature 20: note = May be conjugated to a chemical moiety
  source 1..20: mol_type = other DNA
gtaactgtatttggtacttc

SEQ ID NO: 220 - DNA, 14 bp, synthetic construct
  misc_feature 1..14: note = antisense oligonucleotide
  misc_feature 1: note = May be conjugated to a chemical moiety
  misc_feature 14: note = May be conjugated to a chemical moiety
  source 1..14: mol_type = other DNA
ctgtatttggtact

SEQ ID NO: 221 - DNA, 18 bp, synthetic construct
  misc_feature 1..18: note = antisense oligonucleotide
  source 1..18: mol_type = other DNA
gctattaccttaacccag

SEQ ID NO: 222 - DNA, 18 bp, synthetic construct
  misc_feature 1..18: note = antisense oligonucleotide
  modified_base 1..18: mod_base = OTHER; note = 6 membered morpholine rings replace deoxyribose rings
  misc_feature 1..18: note = linked by non-ionic phosphorodiamidate intersubunit linkages
  misc_feature 18: note = modified with a -C6-NH2 moeity
  source 1..18: mol_type = other DNA
gctattaccttaacccag

SEQ ID NO: 223 - DNA, 18 bp, synthetic construct
  misc_feature 1..18: note = antisense oligonucleotide
  misc_feature 1: note = modified with a cyclooctyne moeity
  modified_base 1..18: mod_base = OTHER; note = 6 membered morpholine rings replace deoxyribose rings
  misc_feature 1..18: note = linked by non-ionic phosphorodiamidate intersubunit linkages
  misc_feature 18: note = modified with a Lissamine Rho moeity
  source 1..18: mol_type = other DNA
gctattaccttaacccag

SEQ ID NO: 224 - DNA, 18 bp, synthetic construct
  misc_feature 1..18: note = antisense oligonucleotide
  misc_feature 1: note = modified with a CPP12-PEG12 moeity
  modified_base 1..18: mod_base = OTHER; note = 6 membered morpholine rings replace deoxyribose rings
  misc_feature 1..18: note = linked by non-ionic phosphorodiamidate intersubunit linkages
  misc_feature 18: note = modified with a Lissamine Rho moeity
  source 1..18: mol_type = other DNA
gctattaccttaacccag

SEQ ID NO: 225 - DNA, 18 bp, synthetic construct
  misc_feature 1..18: note = antisense oligonucleotide
  modified_base 1..18: mod_base = OTHER; note = 6 membered morpholine rings replace deoxyribose rings
  misc_feature 1..18: note = linked by non-ionic phosphorodiamidate intersubunit linkages
  misc_feature 18: note = modified with a CPP12-PEG12-TFP moeity
  source 1..18: mol_type = other DNA
gctattaccttaacccag

SEQ ID NO: 226 - DNA, 18 bp, synthetic construct
  misc_feature 1..18: note = antisense oligonucleotide
  modified_base 1..18: mod_base = OTHER; note = 6 membered morpholine rings replace deoxyribose rings
  misc_feature 1..18: note = linked by non-ionic phosphorodiamidate intersubunit linkages
  misc_feature 18: note = modified with a CPP1212-TFP moeity
  source 1..18: mol_type = other DNA
gctattaccttaacccag

SEQ ID NO: 227 - DNA, 18 bp, synthetic construct
  misc_feature 1..18: note = antisense oligonucleotide
  misc_feature 1: note = modified with a CPP12-(bidentate-no linker)-PEG12 moeity
  modified_base 1..18: mod_base = OTHER; note = 6 membered morpholine rings replace deoxyribose rings
  misc_feature 1..18: note = linked by non-ionic phosphorodiamidate intersubunit linkages
  misc_feature 18: note = modified with a Lissamine Rho moeity
  source 1..18: mol_type = other DNA
gctattaccttaacccag

SEQ ID NO: 228 - DNA, 18 bp, synthetic construct
  misc_feature 1..18: note = antisense oligonucleotide
  misc_feature 1: note = modified with a CPP12-(bidentate-PEG4)-PEG12 moeity
  modified_base 1..18: mod_base = OTHER; note = 6 membered morpholine rings replace deoxyribose rings
  misc_feature 1..18: note = linked by non-ionic phosphorodiamidate intersubunit linkages
  misc_feature 18: note = modified with a Lissamine Rho moeity
  source 1..18: mol_type = other DNA
gctattaccttaacccag

SEQ ID NO: 229 - DNA, 18 bp, synthetic construct
  misc_feature 1..18: note = antisense oligonucleotide
  misc_feature 1: note = modified with a CPP12-(bidentate-PEG12)-PEG12 moeity
  modified_base 1..18: mod_base = OTHER; note = 6 membered morpholine rings replace deoxyribose rings
  misc_feature 1..18: note = linked by non-ionic phosphorodiamidate intersubunit linkages
  misc_feature 18: note = modified with a Lissamine Rho moeity
  source 1..18: mol_type = other DNA
gctattaccttaacccag

SEQ ID NO: 230 - DNA, 18 bp, synthetic construct
  misc_feature 1..18: note = antisense oligonucleotide
  misc_feature 1: note = modified with a CPP12-(tridentate-no linker)-PEG12 moeity
  modified_base 1..18: mod_base = OTHER; note = 6 membered morpholine rings replace deoxyribose rings
  misc_feature 1..18: note = linked by non-ionic phosphorodiamidate intersubunit linkages
  misc_feature 18: note = modified with a Lissamine Rho moeity
  source 1..18: mol_type = other DNA
gctattaccttaacccag

SEQ ID NO: 231 - DNA, 18 bp, synthetic construct
  misc_feature 1..18: note = antisense oligonucleotide
  misc_feature 1: note = modified with a CPP12-(tridentate-PEG4)-PEG12 moeity
  modified_base 1..18: mod_base = OTHER; note = 6 membered morpholine rings replace deoxyribose rings
  misc_feature 1..18: note = linked by non-ionic phosphorodiamidate intersubunit linkages
  misc_feature 18: note = modified with a Lissamine Rho moeity
  source 1..18: mol_type = other DNA
gctattaccttaacccag

SEQ ID NO: 232 - DNA, 18 bp, synthetic construct
  misc_feature 1..18: note = antisense oligonucleotide
  misc_feature 1: note = modified with a CPP12-(tridentate-PEG12)-PEG12 moeity
  modified_base 1..18: mod_base = OTHER; note = 6 membered morpholine rings replace deoxyribose rings
  misc_feature 1..18: note = linked by non-ionic phosphorodiamidate intersubunit linkages
  misc_feature 18: note = modified with a Lissamine Rho moeity
  source 1..18: mol_type = other DNA
gctattaccttaacccag

SEQ ID NO: 233 - DNA, 18 bp, synthetic construct
  misc_feature 1..18: note = antisense oligonucleotide
  modified_base 1..18: mod_base = OTHER; note = 6 membered morpholine rings replace deoxyribose rings
  misc_feature 1..18: note = linked by non-ionic phosphorodiamidate intersubunit linkages
  misc_feature 18: note = modified with a NLS-ss-CPP12 moeity
  source 1..18: mol_type = other DNA
gctattaccttaacccag

SEQ ID NO: 234 - DNA, 18 bp, synthetic construct
  misc_feature 1..18: note = antisense oligonucleotide
  misc_feature 1: note = modified with a Ac-NLS-Lys(CPP12)-PEG12-K(N3) moeity
  modified_base 1..18: mod_base = OTHER; note = 6 membered morpholine rings replace deoxyribose rings
  misc_feature 1..18: note = linked by non-ionic phosphorodiamidate intersubunit linkages
  misc_feature 18: note = modified with a Lissamine Rho moeity
  source 1..18: mol_type = other DNA
gctattaccttaacccag

SEQ ID NO: 235 - DNA, 18 bp, synthetic construct
  misc_feature 1..18: note = antisense oligonucleotide
  modified_base 1..18: mod_base = OTHER; note = 6 membered morpholine rings replace deoxyribose rings
  misc_feature 1..18: note = linked by non-ionic phosphorodiamidate intersubunit linkages
  misc_feature 18: note = modified with a click-K-PEG12-Lys(CPP12)-NLS-Ac moeity
  source 1..18: mol_type = other DNA
gctattaccttaacccag

SEQ ID NO: 236 - DNA, 18 bp, synthetic construct
  misc_feature 1..18: note = antisense oligonucleotide
  modified_base 1..18: mod_base = OTHER; note = 6 membered morpholine rings replace deoxyribose rings
  misc_feature 1..18: note = linked by non-ionic phosphorodiamidate intersubunit linkages
  misc_feature 18: note = modified with a click-Lys(N3)-miniPEG-NLS-ss-PEG12-CPP12 moeity
  source 1..18: mol_type = other DNA
gctattaccttaacccag

SEQ ID NO: 237 - DNA, 25 bp, synthetic construct
  misc_feature 1..25: note = antisense oligonucleotide
  modified_base 1..25: mod_base = OTHER; note = 6 membered morpholine rings replace deoxyribose rings
  misc_feature 1..25: note = linked by non-ionic phosphorodiamidate intersubunit linkages
  source 1..25: mol_type = other DNA
ggccaaacctcggcttacctgaaat

SEQ ID NO: 238 - DNA, 25 bp, synthetic construct
  misc_feature 1..25: note = antisense oligonucleotide
  modified_base 1..25: mod_base = OTHER; note = 6 membered morpholine rings replace deoxyribose rings
  misc_feature 1..25: note = linked by non-ionic phosphorodiamidate intersubunit linkages
  misc_feature 25: note = modified with a C3-NH2 moiety
  source 1..25: mol_type = other DNA
ggccaaacctcggcttacctgaaat

SEQ ID NO: 239 - DNA, 25 bp, synthetic construct
  misc_feature 1..25: note = antisense oligonucleotide
  misc_feature 1: note = modified with a cyclooctyne moiety
  modified_base 1..25: mod_base = OTHER; note = 6 membered morpholine rings replace deoxyribose rings
  misc_feature 1..25: note = linked by non-ionic phosphorodiamidate intersubunit linkages
  source 1..25: mol_type = other DNA
ggccaaacctcggcttacctgaaat

SEQ ID NO: 240 - DNA, 25 bp, synthetic construct
  misc_feature 1..25: note = antisense oligonucleotide
  misc_feature 1: note = modified with a NH2-C3 moiety
  modified_base 1..25: mod_base = OTHER; note = 6 membered morpholine rings replace deoxyribose rings
  misc_feature 1..25: note = linked by non-ionic phosphorodiamidate intersubunit linkages
  misc_feature 25: note = modified with a C3-NH2 moiety
  source 1..25: mol_type = other DNA
ggccaaacctcggcttacctgaaat

SEQ ID NO: 241 - DNA, 25 bp, synthetic construct
  misc_feature 1..25: note = antisense oligonucleotide
  modified_base 1..25: mod_base = OTHER; note = 6 membered morpholine rings replace deoxyribose rings
  misc_feature 1..25: note = linked by non-ionic phosphorodiamidate intersubunit linkages
  misc_feature 25: note = modified with a C4-cyclooctyne moiety
  source 1..25: mol_type = other DNA
ggccaaacctcggcttacctgaaat

SEQ ID NO: 242 - DNA, 25 bp, synthetic construct
  misc_feature 1..25: note = antisense oligonucleotide
  misc_feature 1: note = modified with a CPP12-PEG12-ValCitPABC moiety
  modified_base 1..25: mod_base = OTHER; note = 6 membered morpholine rings replace deoxyribose rings
  misc_feature 1..25: note = linked by non-ionic phosphorodiamidate intersubunit linkages
  source 1..25: mol_type = other DNA
ggccaaacctcggcttacctgaaat

SEQ ID NO: 243 - DNA, 25 bp, synthetic construct
  misc_feature 1..25: note = antisense oligonucleotide
  misc_feature 1: note = modified with a CPP12-PEG12-NH moiety
  modified_base 1..25: mod_base = OTHER; note = 6 membered morpholine rings replace deoxyribose rings
  misc_feature 1..25: note = linked by non-ionic phosphorodiamidate intersubunit linkages
  misc_feature 25: note = modified with a NH-PEG12-CPP12 moiety
  source 1..25: mol_type = other DNA
ggccaaacctcggcttacctgaaat

SEQ ID NO: 244 - DNA, 25 bp, synthetic construct
  misc_feature 1..25: note = antisense oligonucleotide
  modified_base 1..25: mod_base = OTHER; note = 6 membered morpholine rings replace deoxyribose rings
  misc_feature 1..25: note = linked by non-ionic phosphorodiamidate intersubunit linkages
  misc_feature 25: note = modified with a C3-NH-PEG12-CPP12 moiety
  source 1..25: mol_type = other DNA
ggccaaacctcggcttacctgaaat

SEQ ID NO: 245 - DNA, 25 bp, synthetic construct
  misc_feature 1..25: note = antisense oligonucleotide
  misc_feature 1: note = modified with a CPP12-PEG12-Cys-ss-Cys-Lys(N3)-cyclooctyne moiety
  modified_base 1..25: mod_base = OTHER; note = 6 membered morpholine rings replace deoxyribose rings
  misc_feature 1..25: note = linked by non-ionic phosphorodiamidate intersubunit linkages
  source 1..25: mol_type = other DNA
ggccaaacctcggcttacctgaaat

SEQ ID NO: 246 - DNA, 25 bp, synthetic construct
  misc_feature 1..25: note = antisense oligonucleotide
  misc_feature 1: note = modified with a CPP12-PEG12-Lys(N3)-cyclooctyne moiety
  modified_base 1..25: mod_base = OTHER; note = 6 membered morpholine rings replace deoxyribose rings
  misc_feature 1..25: note = linked by non-ionic phosphorodiamidate intersubunit linkages
  source 1..25: mol_type = other DNA
ggccaaacctcggcttacctgaaat

SEQ ID NO: 247 - DNA, 25 bp, synthetic construct
  misc_feature 1..25: note = antisense oligonucleotide
  misc_feature 1: note = modified with a CPP12-PEG12-Prodisulfide moiety
  modified_base 1..25: mod_base = OTHER; note = 6 membered morpholine rings replace deoxyribose rings
  misc_feature 1..25: note = linked by non-ionic phosphorodiamidate intersubunit linkages
  source 1..25: mol_type = other DNA
ggccaaacctcggcttacctgaaat

SEQ ID NO: 248 - DNA, 25 bp, synthetic construct
  misc_feature 1..25: note = antisense oligonucleotide
  misc_feature 1: note = modified with a CPP12-PEG24 moiety
  modified_base 1..25: mod_base = OTHER; note = 6 membered morpholine rings replace deoxyribose rings
  misc_feature 1..25: note = linked by non-ionic phosphorodiamidate intersubunit linkages
  source 1..25: mol_type = other DNA
ggccaaacctcggcttacctgaaat

SEQ ID NO: 249 - DNA, 25 bp, synthetic construct
  misc_feature 1..25: note = antisense oligonucleotide
  modified_base 1..25: mod_base = OTHER; note = 6 membered morpholine rings replace deoxyribose rings
  misc_feature 1..25: note = linked by non-ionic phosphorodiamidate intersubunit linkages
  misc_feature 25: note = modified with a C3NH-C6-CPP12 moiety
  source 1..25: mol_type = other DNA
ggccaaacctcggcttacctgaaat

SEQ ID NO: 250 - DNA, 25 bp, synthetic construct
  misc_feature 1..25: note = antisense oligonucleotide
  misc_feature 1: note = modified with a CPP12-(bidentate-no linker)-PEG12 moiety
  modified_base 1..25: mod_base = OTHER; note = 6 membered morpholine rings replace deoxyribose rings
  misc_feature 1..25: note = linked by non-ionic phosphorodiamidate intersubunit linkages
  source 1..25: mol_type = other DNA
ggccaaacctcggcttacctgaaat

SEQ ID NO: 251 - DNA, 25 bp, synthetic construct
  misc_feature 1..25: note = antisense oligonucleotide
  misc_feature 1: note = modified with a CPP12-(bidentate-PEG12)-PEG12 moiety
  modified_base 1..25: mod_base = OTHER; note = 6 membered morpholine rings replace deoxyribose rings
  misc_feature 1..25: note = linked by non-ionic phosphorodiamidate intersubunit linkages
  source 1..25: mol_type = other DNA
ggccaaacctcggcttacctgaaat

SEQ ID NO: 252 - DNA, 25 bp, synthetic construct
  misc_feature 1..25: note = antisense oligonucleotide
  modified_base 1..25: mod_base = OTHER; note = 6 membered morpholine rings replace deoxyribose rings
  misc_feature 1..25: note = linked by non-ionic phosphorodiamidate intersubunit linkages
  misc_feature 25: note = modified with a C3-NH-CPP1212 moiety
  source 1..25: mol_type = other DNA
ggccaaacctcggcttacctgaaat

SEQ ID NO: 253 - DNA, 25 bp, synthetic construct
  misc_feature 1..25: note = antisense oligonucleotide
  misc_feature 1: note = modified with a T9-PEG12-CPP12-PEG12 moiety
  modified_base 1..25: mod_base = OTHER; note = 6 membered morpholine rings replace deoxyribose rings
  misc_feature 1..25: note = linked by non-ionic phosphorodiamidate intersubunit linkages
  source 1..25: mol_type = other DNA
ggccaaacctcggcttacctgaaat

SEQ ID NO: 254 - DNA, 25 bp, synthetic construct
  misc_feature 1..25: note = antisense oligonucleotide
  misc_feature 1: note = modified with a Ac-MSP-PEG12-Lys(CPP12-PEG12)-K(N3) moiety
  modified_base 1..25: mod_base = OTHER; note = 6 membered morpholine rings replace deoxyribose rings
  misc_feature 1..25: note = linked by non-ionic phosphorodiamidate intersubunit linkages
  source 1..25: mol_type = other DNA
ggccaaacctcggcttacctgaaat

SEQ ID NO: 255 - DNA, 25 bp, synthetic construct
  misc_feature 1..25: note = antisense oligonucleotide
  modified_base 1..25: mod_base = OTHER; note = 6 membered morpholine rings replace deoxyribose rings
  misc_feature 1..25: note = linked by non-ionic phosphorodiamidate intersubunit linkages
  misc_feature 25: note = modified with a C3NH-PEG4-BCN+Lys(N3)-miniPEG-NLS-ss-bA-bA-CPP12 moiety
  source 1..25: mol_type = other DNA
ggccaaacctcggcttacctgaaat

SEQ ID NO: 256 - DNA, 25 bp, synthetic construct
  misc_feature 1..25: note = antisense oligonucleotide
  modified_base 1..25: mod_base = OTHER; note = 6 membered morpholine rings replace deoxyribose rings
  misc_feature 1..25: note = linked by non-ionic phosphorodiamidate intersubunit linkages
  misc_feature 25: note = modified with a C3NH-PEG4-BCN+Ac-NLS-Lys(CPP12)-PEG12-K(N3) moiety
  source 1..25: mol_type = other DNA
ggccaaacctcggcttacctgaaat

SEQ ID NO: 257 - DNA, 25 bp, synthetic construct
  misc_feature 1..25: note = antisense oligonucleotide
  modified_base 1..25: mod_base = OTHER; note = 6 membered morpholine rings replace deoxyribose rings
  misc_feature 1..25: note = linked by non-ionic phosphorodiamidate intersubunit linkages
  misc_feature 25: note = modified with a click-K-PEG12-Lys(CPP12)-NLS-Ac moiety
  source 1..25: mol_type = other DNA
ggccaaacctcggcttacctgaaat

SEQ ID NO: 258 - protein, 12 aa, synthetic construct
  REGION 1..12: note = T9 peptide
SKTFNTHPQSTP

SEQ ID NO: 259 - protein, 7 aa, synthetic construct
  REGION 1..7: note = MSP peptide
ASSLNIA

SEQ ID NO: 260 - DNA, 25 bp, synthetic construct
  misc_feature 1..25: note = antisense oligonucleotide
  source 1..25: mol_type = other DNA
ggccaaacctcggcttacctgaaat

SEQ ID NO: 261 - DNA, 22 bp, synthetic construct
  misc_feature 1..22: note = oligonucleotide primer
  source 1..22: mol_type = other DNA
cagaattctgccaattgctgag

SEQ ID NO: 262 - DNA, 20 bp, synthetic construct
  misc_feature 1..20: note = oligonucleotide primer
  source 1..20: mol_type = other DNA
ttcttcagcttgtgtcatcc

SEQ ID NO: 263 - DNA, 24 bp, synthetic construct
  misc_feature 1..24: note = oligonucleotide primer
  source 1..24: mol_type = other DNA
cccagtctaccaccctatcagagc

SEQ ID NO: 264 - DNA, 20 bp, synthetic construct
  misc_feature 1..20: note = oligonucleotide primer
  source 1..20: mol_type = other DNA
cctgcctttaaggcttcctt

SEQ ID NO: 265 - DNA, 21 bp, synthetic construct
  misc_feature 1..21: note = antisense oligonucleotide
  modified_base 1..21: mod_base = OTHER; note = 6 membered morpholine rings replace deoxyribose rings
  misc_feature 1..21: note = linked by non-ionic phosphorodiamidate intersubunit linkages
  misc_feature 21: note = modified with a primary amine moiety
  source 1..21: mol_type = other DNA
gtaactgtatttggtacttcc

SEQ ID NO: 266 - DNA, 21 bp, synthetic construct
  misc_feature 1..21: note = antisense oligonucleotide
  modified_base 1..21: mod_base = OTHER; note = 6 membered morpholine rings replace deoxyribose rings
  misc_feature 1..21: note = linked by non-ionic phosphorodiamidate intersubunit linkages
  misc_feature 21: note = modified with a PEG12CPP12 moiety
  source 1..21: mol_type = other DNA
gtaactgtatttggtacttcc

SEQ ID NO: 267 - DNA, 15 bp, synthetic construct
  misc_feature 1..15: note = antisense oligonucleotide
  modified_base 1..15: mod_base = OTHER; note = 6 membered morpholine rings replace deoxyribose rings
  misc_feature 1..15: note = linked by non-ionic phosphorodiamidate intersubunit linkages
  misc_feature 15: note = modified with a CPP12-PEG12-K(CPP12)-PEG12-TFP moiety
  source 1..15: mol_type = other DNA
ctgtatttggtactt

SEQ ID NO: 268 - DNA, 21 bp, synthetic construct
  misc_feature 1..21: note = antisense oligonucleotide
  modified_base 1..21: mod_base = OTHER; note = 6 membered morpholine rings replace deoxyribose rings
  misc_feature 1..21: note = linked by non-ionic phosphorodiamidate intersubunit linkages
  misc_feature 21: note = modified with a CPP12-PEG12-K(CPP12)-PEG12-TFP moiety
  source 1..21: mol_type = other DNA
gtaactgtatttggtacttcc

SEQ ID NO: 269 - DNA, 21 bp, synthetic construct
  misc_feature 1..21: note = antisense oligonucleotide
  modified_base 1..21: mod_base = OTHER; note = 6 membered morpholine rings replace deoxyribose rings
  misc_feature 1..21: note = linked by non-ionic phosphorodiamidate intersubunit linkages
  misc_feature 21: note = modified with a Ac-NLS-Lys(CPP12)-PEG12-K(N3) moiety
  source 1..21: mol_type = other DNA
gtaactgtatttggtacttcc

SEQ ID NO: 270 - DNA, 15 bp, Homo sapiens
  source 1..15: mol_type = other DNA
ctgtatttggtactt

SEQ ID NO: 271 - DNA, 18 bp, synthetic construct
  misc_feature 1..18: note = oligonucleotide primer
  source 1..18: mol_type = other DNA
ctcagacatgccgctgct

SEQ ID NO: 272 - DNA, 22 bp, synthetic construct
  misc_feature 1..22: note = oligonucleotide primer
  source 1..22: mol_type = other DNA
ttgagctggatggttctctccg